European Patent Application EP 4 144 763 A1, published March 8, 2023. Title: BIFUNCTIONAL PROTEIN AGAINST PD-1 AND TGF-β. Applicant: Chia Tai Tianqing Pharmaceutical Group Co., Ltd. The sequence listing filed with the application follows.

SEQUENCE LISTING (22 sequences)

SEQ ID NO: 1 - protein, 8 aa, Artificial Sequence
  HCDR1 of anti-PD-1 antibody
GFAFSSYD

SEQ ID NO: 2 - protein, 8 aa, Artificial Sequence
  HCDR2 of anti-PD-1 antibody
ISGGGRYT

SEQ ID NO: 3 - protein, 11 aa, Artificial Sequence
  HCDR3 of anti-PD-1 antibody
ANRYGEAWFAY

SEQ ID NO: 4 - protein, 6 aa, Artificial Sequence
  LCDR1 of anti-PD-1 antibody
QDINTY

SEQ ID NO: 5 - protein, 3 aa, Artificial Sequence
  LCDR2 of anti-PD-1 antibody
RAN

SEQ ID NO: 6 - protein, 9 aa, Artificial Sequence
  LCDR3 of anti-PD-1 antibody
LQYDEFPLT

SEQ ID NO: 7 - protein, 118 aa, Artificial Sequence
  VH of anti-PD-1 antibody
EVQLVESGGGLVQPGGSLRLSCAASGFAFSSYDMSWVRQAPGKGLDWVATISGGGRYTYYPDSVKGRFTISRDNSKNNLYLQMNSLRAEDTALYYCANRYGEAWFAYWGQGTLVTVSS

SEQ ID NO: 8 - protein, 107 aa, Artificial Sequence
  VL of anti-PD-1 antibody
DIQMTQSPSSMSASVGDRVTFTCRASQDINTYLSWFQQKPGKSPKTLIYRANRLVSGVPSRFSGSGSGQDYTLTISSLQPEDMATYYCLQYDEFPLTFGAGTKLELK

SEQ ID NO: 9 - protein, 330 aa, Artificial Sequence
  Heavy chain constant region of anti-PD-1 antibody
ASTKGPSVFPLAPSSKSTSGGTAALGCLVKDYFPEPVTVSWNSGALTSGVHTFPAVLQSSGLYSLSSVVTVPSSSLGTQTYICNVNHKPSNTKVDKKVEPKSCDKTHTCPPCPAPEAAGAPSVFLFPPKPKDTLMISRTPEVTCVVVDVSHEDPEVKFNWYVDGVEVHNAKTKPREEQYNSTYRVVSVLTVLHQDWLNGKEYKCKVSNKALPAPIEKTISKAKGQPREPQVYTLPPSRDELTKNQVSLTCLVKGFYPSDIAVEWESNGQPENNYKTTPPVLDSDGSFFLYSKLTVDKSRWQQGNVFSCSVMHEALHNHYTQKSLSLSPGA

SEQ ID NO: 10 - protein, 107 aa, Artificial Sequence [sequence omitted]

SEQ ID NO: 11 - protein, 136 aa, Homo sapiens
IPPHVQKSVNNDMIVTDNNGAVKFPQLCKFCDVRFSTCDNQKSCMSNCSITSICEKPQEVCVAVWRKNDENITLETVCHDPKLPYHDFILEDAASPKCIMKEKKKPGETFFMCSCSSDECNDNIIFSEEYNTSNPD

SEQ ID NO: 12 - protein, 21 aa, Artificial Sequence
  flexible linker
GGGGSGGGGSGGGGSGGGGSG

SEQ ID NO: 13 - protein, 605 aa, Artificial Sequence
  heavy chain portion of PD-1/TGFβ bifunctional protein
EVQLVESGGGLVQPGGSLRLSCAASGFAFSSYDMSWVRQAPGKGLDWVATISGGGRYTYYPDSVKGRFTISRDNSKNNLYLQMNSLRAEDTALYYCANRYGEAWFAYWGQGTLVTVSSASTKGPSVFPLAPSSKSTSGGTAALGCLVKDYFPEPVTVSWNSGALTSGVHTFPAVLQSSGLYSLSSVVTVPSSSLGTQTYICNVNHKPSNTKVDKKVEPKSCDKTHTCPPCPAPEAAGAPSVFLFPPKPKDTLMISRTPEVTCVVVDVSHEDPEVKFNWYVDGVEVHNAKTKPREEQYNSTYRVVSVLTVLHQDWLNGKEYKCKVSNKALPAPIEKTISKAKGQPREPQVYTLPPSRDELTKNQVSLTCLVKGFYPSDIAVEWESNGQPENNYKTTPPVLDSDGSFFLYSKLTVDKSRWQQGNVFSCSVMHEALHNHYTQKSLSLSPGAGGGGSGGGGSGGGGSGGGGSGIPPHVQKSVNNDMIVTDNNGAVKFPQLCKFCDVRFSTCDNQKSCMSNCSITSICEKPQEVCVAVWRKNDENITLETVCHDPKLPYHDFILEDAASPKCIMKEKKKPGETFFMCSCSSDECNDNIIFSEEYNTSNPD

SEQ ID NO: 14 - protein, 214 aa, Artificial Sequence
  light chain portion of PD-1/TGFβ bifunctional protein
DIQMTQSPSSMSASVGDRVTFTCRASQDINTYLSWFQQKPGKSPKTLIYRANRLVSGVPSRFSGSGSGQDYTLTISSLQPEDMATYYCLQYDEFPLTFGAGTKLELKRTVAAPSVFIFPPSDEQLKSGTASVVCLLNNFYPREAKVQWKVDNALQSGNSQESVTEQDSKDSTYSLSSTLTLSKADYEKHKVYACEVTHQGLSSPVTKSFNRGEC

SEQ ID NO: 15 - DNA, 1815 bp, Artificial Sequence
  encoding sequence of heavy chain portion of PD-1/TGFβ bifunctional protein
gaggtacaactggtggaatccggtggcggtctcgtgcagcctggcggcagcctgagactgagttgtgctgcttctggctttgccttctcctcctacgacatgtcctgggtgcggcaggcccctggaaagggcctggattgggtggccaccatttccggaggcggcagatacacctactaccctgactctgtcaagggccggttcaccatctccagagacaactccaagaacaacctgtacctgcagatgaactccctgagagccgaggacaccgccctgtactactgcgccaaccggtacggcgaggcttggttcgcctactggggccaaggcaccctcgtgaccgtatcatccgcctccacaaagggcccttctgtgttccctctggccccttcctccaagtctacaagcggaggcaccgctgctctgggctgcctggtcaaggactacttccccgaacccgtgaccgtgtcttggaactccggcgctctgacctctggagtgcataccttccctgccgtgctgcagtcctccggcctgtactctctgtccagcgtggtcaccgtgcctagcagcagtctgggaacccagacatacatctgcaacgtgaaccacaagccctccaatacaaaagtggacaagaaggtggagcctaaatcctgcgacaagacccacacctgtcctccttgccctgctcctgaggccgctggcgccccttctgtgtttctgttcccccctaagcccaaggacaccctgatgatctcccggacccccgaggtgacctgcgtggtggtggacgtgtcccacgaggaccctgaagtgaagttcaactggtacgtggatggcgtggaagtgcacaacgccaagaccaagcctagagaggagcagtacaacagcacctacagagtggtctccgtgctgaccgttctgcaccaggactggctgaacggcaaggagtacaagtgcaaggtgtccaacaaggccctgcccgcccctatcgagaagaccatctctaaggctaagggccagcctagagaacctcaagtgtacaccctgcctccatctcgggatgagctgacaaagaatcaggtgtctctgacctgtctggtgaagggcttctacccctctgacatcgccgtggagtgggagtctaacggccagcccgagaacaactacaagaccacccctcctgtgctggactccgacggctccttcttcctgtactccaagctgaccgtggacaagtctagatggcagcagggcaacgtgttctcctgctccgtgatgcacgaggccctgcacaaccactacacacagaaatccctgtccctgtcccctggcgctggaggcggtggctccggcggcggcggctccggtggcggaggctccggaggcggcggctctggcatcccccctcacgtgcagaagagcgtcaacaacgatatgatcgtgaccgacaacaacggagctgtgaagtttcctcaactgtgcaagttctgcgacgtcagattctctacctgtgataaccagaagtcctgcatgtccaactgcagcatcacctccatctgcgagaaacctcaagaggtgtgcgtggctgtgtggcggaagaacgacgaaaacatcaccctggaaaccgtatgtcacgatcctaagctgccttaccacgacttcatcctggaagatgccgcctctcccaagtgcatcatgaaagagaagaagaaacccggcgagacctttttcatgtgctcttgctccagcgacgagtgcaacgacaatatcatcttcagcgaggaatacaacaccagcaaccctgac

SEQ ID NO: 16 - DNA, 642 bp, Artificial Sequence
  encoding sequence of light chain portion of PD-1/TGFβ bifunctional protein
gatatccagatgacccagtccccctcctccatgtccgcctccgtgggcgacagagtgaccttcacctgcagagcttctcaggacatcaacacctacctgtcctggttccagcagaagcctggcaagtctcctaagaccctgatctacagagccaaccggctggtgtccggcgtgccttctcggttctccggatctggctctggccaggattacaccctgaccatctcctctctgcagcctgaggacatggccacctactactgcctgcagtacgacgagttccctctgacattcggcgctggcaccaagctggaactgaagcggaccgtggccgctcctagcgtgttcatcttccctccttccgacgaacaactgaagtccggcaccgcctctgtggtgtgcctgctgaacaacttctaccctagagaggccaaggtgcagtggaaggtggacaacgccctgcaaagcggcaactcccaagagtccgtcaccgagcaggacagcaaggactccacctactccctgtcttctacactgaccctgtccaaggccgactacgagaagcacaaggtgtacgcctgcgaggtgacacaccagggcctgagctcccctgtgaccaagtccttcaacagaggcgagtgc

SEQ ID NO: 17 - protein, 440 aa, Artificial Sequence
  heavy chain of Nivolumab
QVQLVESGGGVVQPGRSLRLDCKASGITFSNSGMHWVRQAPGKGLEWVAVIWYDGSKRYYADSVKGRFTISRDNSKNTLFLQMNSLRAEDTAVYYCATNDDYWGQGTLVTVSSASTKGPSVFPLAPCSRSTSESTAALGCLVKDYFPEPVTVSWNSGALTSGVHTFPAVLQSSGLYSLSSVVTVPSSSLGTKTYTCNVDHKPSNTKVDKRVESKYGPPCPPCPAPEFLGGPSVFLFPPKPKDTLMISRTPEVTCVVVDVSQEDPEVQFNWYVDGVEVHNAKTKPREEQFNSTYRVVSVLTVLHQDWLNGKEYKCKVSNKGLPSSIEKTISKAKGQPREPQVYTLPPSQEEMTKNQVSLTCLVKGFYPSDIAVEWESNGQPENNYKTTPPVLDSDGSFFLYSRLTVDKSRWQEGNVFSCSVMHEALHNHYTQKSLSLSLGK

SEQ ID NO: 18 - protein, 214 aa, Artificial Sequence
  light chain of Nivolumab
EIVLTQSPATLSLSPGERATLSCRASQSVSSYLAWYQQKPGQAPRLLIYDASNRATGIPARFSGSGSGTDFTLTISSLEPEDFAVYYCQQSSNWPRTFGQGTKVEIKRTVAAPSVFIFPPSDEQLKSGTASVVCLLNNFYPREAKVQWKVDNALQSGNSQESVTEQDSKDSTYSLSSTLTLSKADYEKHKVYACEVTHQGLSSPVTKSFNRGEC

SEQ ID NO: 19 - protein, 448 aa, Artificial Sequence
  heavy chain of PD1 monoclonal antibody in CN106977602
EVQLVESGGGLVQPGGSLRLSCAASGFAFSSYDMSWVRQAPGKGLDWVATISGGGRYTYYPDSVKGRFTISRDNSKNNLYLQMNSLRAEDTALYYCANRYGEAWFAYWGQGTLVTVSSASTKGPSVFPLAPSSKSTSGGTAALGCLVKDYFPEPVTVSWNSGALTSGVHTFPAVLQSSGLYSLSSVVTVPSSSLGTQTYICNVNHKPSNTKVDKKVEPKSCDKTHTCPPCPAPEAAGAPSVFLFPPKPKDTLMISRTPEVTCVVVDVSHEDPEVKFNWYVDGVEVHNAKTKPREEQYNSTYRVVSVLTVLHQDWLNGKEYKCKVSNKALPAPIEKTISKAKGQPREPQVYTLPPSRDELTKNQVSLTCLVKGFYPSDIAVEWESNGQPENNYKTTPPVLDSDGSFFLYSKLTVDKSRWQQGNVFSCSVMHEALHNHYTQKSLSLSPGK

SEQ ID NO: 20 - protein, 597 aa, Artificial Sequence
  heavy chain portion of Nivolumab/TGF-βRII bifunctional protein
QVQLVESGGGVVQPGRSLRLDCKASGITFSNSGMHWVRQAPGKGLEWVAVIWYDGSKRYYADSVKGRFTISRDNSKNTLFLQMNSLRAEDTAVYYCATNDDYWGQGTLVTVSSASTKGPSVFPLAPCSRSTSESTAALGCLVKDYFPEPVTVSWNSGALTSGVHTFPAVLQSSGLYSLSSVVTVPSSSLGTKTYTCNVDHKPSNTKVDKRVESKYGPPCPPCPAPEFLGGPSVFLFPPKPKDTLMISRTPEVTCVVVDVSQEDPEVQFNWYVDGVEVHNAKTKPREEQFNSTYRVVSVLTVLHQDWLNGKEYKCKVSNKGLPSSIEKTISKAKGQPREPQVYTLPPSQEEMTKNQVSLTCLVKGFYPSDIAVEWESNGQPENNYKTTPPVLDSDGSFFLYSRLTVDKSRWQEGNVFSCSVMHEALHNHYTQKSLSLSLGAGGGGSGGGGSGGGGSGGGGSGIPPHVQKSVNNDMIVTDNNGAVKFPQLCKFCDVRFSTCDNQKSCMSNCSITSICEKPQEVCVAVWRKNDENITLETVCHDPKLPYHDFILEDAASPKCIMKEKKKPGETFFMCSCSSDECNDNIIFSEEYNTSNPD

SEQ ID NO: 21 - protein, 446 aa, Artificial Sequence
  heavy chain of IgG1 protein
EVQLEQSGAELMKPGASVKISCKATGYTFTTYWIEWIKQRPGHSLEWIGEILPGSDSTYYNEKVKGKVTFTADASSNTAYMQLSSLTSEDSAVYYCARGDGFYVYWGQGTTLTVSSASTKGPSVFPLAPSSKSTSGGTAALGCLVKDYFPEPVTVSWNSGALTSGVHTFPAVLQSSGLYSLSSVVTVPSSSLGTQTYICNVNHKPSNTKVDKKVEPKSCDKTHTCPPCPAPELLGGPSVFLFPPKPKDTLMISRTPEVTCVVVDVSHEDPEVKFNWYVDGVEVHNAKTKPREEQYNSTYRVVSVLTVLHQDWLNGKEYKCKVSNKALPAPIEKTISKAKGQPREPQVYTLPPSRDELTKNQVSLTCLVKGFYPSDIAVEWESNGQPENNYKTTPPVLDSDGSFFLYSKLTVDKSRWQQGNVFSCSVMHEALHNHYTQKSLSLSPGK

SEQ ID NO: 22 - protein, 214 aa, Artificial Sequence
  light chain of IgG1 protein
DIELTQSPATLSVTPGDSVSLSCRASQSISNNLHWYQQKSHESPRLLIKYTSQSMSGIPSRFSGSGSGTDFTLSINSVETEDFGVYFCQQSGSWPRTFGGGTKLDIKRTVAAPSVFIFPPSDEQLKSGTASVVCLLNNFYPREAKVQWKVDNALQSGNSQESVTEQDSKDSTYSLSSTLTLSKADYEKHKVYACEVTHQGLSSPVTKSFNRGEC